European Patent Specification EP 3 755 813 B1, published August 9, 2023. Title: IMPROVED DETECTION OF MICROSATELLITE INSTABILITY. Applicant: Roche Diagnostics GmbH F. Hoffmann-La Roche AG Roche Molecular Systems, Inc. The sequence listing filed with the application follows.

SEQUENCE LISTING (28 sequences)

SEQ ID NO: 1 - DNA, 31 bp, Artificial Sequence
  source: /note="Description of Artificial Sequence: Synthetic oligonucleotide"
tgatttttttttttttttttttttttttgag

SEQ ID NO: 2 - DNA, 36 bp, Artificial Sequence
  source: /note="Description of Artificial Sequence: Synthetic oligonucleotide"
  misc_feature (17)..(36): /note="This region may encompass 16-20 nucleotides"
aaaaaaaaaaaaaaaaaaaaaaaaaaaaaaaaaaaa

SEQ ID NO: 3 - DNA, 38 bp, Artificial Sequence
  source: /note="Description of Artificial Sequence: Synthetic oligonucleotide"
ctgatttttttttttttttttttttttttgagaatcag

SEQ ID NO: 4 - DNA, 31 bp, Artificial Sequence; identical to SEQ ID NO: 1
  source: /note="Description of Artificial Sequence: Synthetic oligonucleotide"

SEQ ID NO: 5 - DNA, 32 bp, Artificial Sequence
  source: /note="Description of Artificial Sequence: Synthetic oligonucleotide"
cctttttttttttttttttttttttttttacc

SEQ ID NO: 6 - DNA, 30 bp, Artificial Sequence
  source: /note="Description of Artificial Sequence: Synthetic oligonucleotide"
ccttttttttttttttttttttttagcaac

SEQ ID NO: 7 - DNA, 34 bp, Artificial Sequence
  source: /note="Description of Artificial Sequence: Synthetic oligonucleotide"
tcctattttttttttttttttttttttttgtgag

SEQ ID NO: 8 - DNA, 34 bp, Artificial Sequence
  source: /note="Description of Artificial Sequence: Synthetic oligonucleotide"
actctttttttttttttttttttttttttttgag

SEQ ID NO: 9 - DNA, 31 bp, Artificial Sequence
  source: /note="Description of Artificial Sequence: Synthetic oligonucleotide"
tggccttttttttttttttttttttttagca

SEQ ID NO: 10 - DNA, 46 bp, Artificial Sequence
  source: /note="Description of Artificial Sequence: Synthetic oligonucleotide"
  modified_base (5)..(5): a, c, t, g, unknown or other
  modified_base (7)..(7): a, c, t, g, unknown or other
  modified_base (12)..(12): a, c, t, g, unknown or other
  modified_base (20)..(20): a, c, t, g, unknown or other
ttttntnttttntttttttnattttttttttttttttttttttttt

SEQ ID NO: 11 - DNA, 37 bp, Artificial Sequence
  source: /note="Description of Artificial Sequence: Synthetic oligonucleotide"
  modified_base (6)..(11): a, c, t, g, unknown or other
tttttnnnnnnaaaaaaaaaaaaaaaaaaaaaaaaaa

SEQ ID NO: 12 - DNA, 21 bp, Artificial Sequence
  source: /note="Description of Artificial Sequence: Synthetic oligonucleotide"
ttttttttttttttttttttt

SEQ ID NO: 13 - DNA, 24 bp, Artificial Sequence
  source: /note="Description of Artificial Sequence: Synthetic oligonucleotide"
tttttttttttttttttttttttt

SEQ ID NO: 14 - DNA, 27 bp, Artificial Sequence
  source: /note="Description of Artificial Sequence: Synthetic oligonucleotide"
aaaaaaaaaaaaaaaaaaaaaaaaaaa

SEQ ID NO: 15 - DNA, 71 bp, Artificial Sequence
  source: /note="Description of Artificial Sequence: Synthetic oligonucleotide"
  modified_base (5)..(5): a, c, t, g, unknown or other
  modified_base (8)..(9): a, c, t, g, unknown or other
  modified_base (17)..(26): a, c, t, g, unknown or other
  modified_base (31)..(31): a, c, t, g, unknown or other
ttttnttnntttttttnnnnnnnnnnttttntttttttttttttttttttttttttttttttttttttttt

SEQ ID NO: 16 - DNA, 72 bp, Artificial Sequence
  source: /note="Description of Artificial Sequence: Synthetic oligonucleotide"
  misc_feature (59)..(72): /note="This region may encompass 'ttttttt' or 'gagagagagagaga' wherein some positions may be absent"
cacacacacacacacacacacacacatacacacacacacacacacacacacacacacannnnnnnnnnnnnn

SEQ ID NO: 17 - DNA, 52 bp, Artificial Sequence
  source: /note="Description of Artificial Sequence: Synthetic oligonucleotide"
cacacacacacacacacacacacacacacacacacacacacacacacacaca

SEQ ID NO: 18 - DNA, 87 bp, Artificial Sequence
  source: /note="Description of Artificial Sequence: Synthetic oligonucleotide"
  modified_base (15)..(39): a, c, t, g, unknown or other
tatatatatatatannnnnnnnnnnnnnnnnnnnnnnnncacacacacacacacacacacacacacacacacacacacacacacaca

SEQ ID NO: 19 - DNA, 75 bp, Artificial Sequence
  source: /note="Description of Artificial Sequence: Synthetic oligonucleotide"
  misc_feature (1)..(75): /note="This sequence may encompass 3-15 'aaaag' repeating units"
aaaagaaaagaaaagaaaagaaaagaaaagaaaagaaaagaaaagaaaagaaaagaaaagaaaagaaaagaaaag

SEQ ID NO: 20 - DNA, 85 bp, Artificial Sequence
  source: /note="Description of Artificial Sequence: Synthetic oligonucleotide"
  misc_feature (1)..(85): /note="This sequence may encompass 2-17 'aaaag' repeating units"
aaaagaaaagaaaagaaaagaaaagaaaagaaaagaaaagaaaagaaaagaaaagaaaagaaaagaaaagaaaagaaaagaaaag

SEQ ID NO: 21 - DNA, 149 bp, Artificial Sequence
  source: /note="Description of Artificial Sequence: Synthetic polynucleotide"
gaaaagaaagaaataaarrrrrrrrrrgaaagagaaagaaagaaagaaagaaagaaagaaagaaagaaagaaagaaagaaagaaagaaagaaagaaaagaaaagaaaagaaaagaaaagaaaagaaaagaaaagaaaaagaaaagaaaa

SEQ ID NO: 22 - DNA, 33 bp, Artificial Sequence
  source: /note="Description of Artificial Sequence: Synthetic oligonucleotide"
tttgatttttttttttttttttttttttttacc

SEQ ID NO: 23 - DNA, 22 bp, Artificial Sequence
  source: /note="Description of Artificial Sequence: Synthetic oligonucleotide"
tttttttttttttttttttttt

SEQ ID NO: 24 - DNA, 25 bp, Artificial Sequence
  source: /note="Description of Artificial Sequence: Synthetic oligonucleotide"
ttttttttttttttttttttttttt

SEQ ID NO: 25 - DNA, 18 bp, Artificial Sequence
  source: /note="Description of Artificial Sequence: Synthetic oligonucleotide"
tttttttttttttttttt

SEQ ID NO: 26 - DNA, 27 bp, Artificial Sequence
  source: /note="Description of Artificial Sequence: Synthetic oligonucleotide"
ttttttttttttttttttttttttttt

SEQ ID NO: 27 - DNA, 16 bp, Artificial Sequence
  source: /note="Description of Artificial Sequence: Synthetic oligonucleotide"
aaaaaaaaaaaaaaaa

SEQ ID NO: 28 - DNA, 12 bp, Artificial Sequence
  source: /note="Description of Artificial Sequence: Synthetic oligonucleotide"
aaaaaaaaaaaa